European Patent Application EP 4 763 969 A1, published June 24, 2026. Title: Bone-on-Chip Microfluidic Device. Applicant: CanChip GmbH. The sequence listing filed with the application follows.

SEQUENCE LISTING (44 sequences)

SEQ ID NO: 1 - DNA, 21 bp, synthetic construct
  source 1..21: mol_type = other DNA; note = primer
atctttggtctggcccccatg

SEQ ID NO: 2 - DNA, 23 bp, synthetic construct
  source 1..23: mol_type = other DNA; note = primer
agtccaccatggagcattctctc

SEQ ID NO: 3 - DNA, 22 bp, synthetic construct
  source 1..22: mol_type = other DNA; note = primer
caaccacagaaccacaagtgcg

SEQ ID NO: 4 - DNA, 22 bp, synthetic construct
  source 1..22: mol_type = other DNA; note = primer
tgtttgatgccatagtccctcc

SEQ ID NO: 5 - DNA, 20 bp, synthetic construct
  source 1..20: mol_type = other DNA; note = primer
tcacactcctcgccctattg

SEQ ID NO: 6 - DNA, 20 bp, synthetic construct
  source 1..20: mol_type = other DNA; note = primer
gaagaggaaagaagggtgcc

SEQ ID NO: 7 - DNA, 20 bp, synthetic construct
  source 1..20: mol_type = other DNA; note = primer
cgaatacacgggcgtcaatg

SEQ ID NO: 8 - DNA, 23 bp, synthetic construct
  source 1..23: mol_type = other DNA; note = primer
gtagctgtactcatcttcatggc

SEQ ID NO: 9 - DNA, 27 bp, synthetic construct
  source 1..27: mol_type = other DNA; note = primer
tcaccagtctgatgagtctcaccattc

SEQ ID NO: 10 - DNA, 26 bp, synthetic construct
  source 1..26: mol_type = other DNA; note = primer
tagcatcagggtactggatgtcaggt

SEQ ID NO: 11 - DNA, 21 bp, synthetic construct
  source 1..21: mol_type = other DNA; note = primer
agggcagaatcatcacgaagt

SEQ ID NO: 12 - DNA, 20 bp, synthetic construct
  source 1..20: mol_type = other DNA; note = primer
agggtctcgattggatggca

SEQ ID NO: 13 - DNA, 18 bp, synthetic construct
  source 1..18: mol_type = other DNA; note = primer
taaagggtcaccgtggct

SEQ ID NO: 14 - DNA, 18 bp, synthetic construct
  source 1..18: mol_type = other DNA; note = primer
cgaaccacattgccatca

SEQ ID NO: 15 - DNA, 20 bp, synthetic construct
  source 1..20: mol_type = other DNA; note = primer
ccatccaatcggtagtagcg

SEQ ID NO: 16 - DNA, 20 bp, synthetic construct
  source 1..20: mol_type = other DNA; note = primer
gtaacccgttgaaccccatt

SEQ ID NO: 17 - DNA, 20 bp, synthetic construct
  source 1..20: mol_type = other DNA; note = primer
gccgaggtgatagtgtggtt

SEQ ID NO: 18 - DNA, 23 bp, synthetic construct
  source 1..23: mol_type = other DNA; note = primer
tgaggtgatgtcctcgtcgtctg

SEQ ID NO: 19 - DNA, 20 bp, synthetic construct
  source 1..20: mol_type = other DNA; note = primer
agccttgccttgctgctcta

SEQ ID NO: 20 - DNA, 18 bp, synthetic construct
  source 1..18: mol_type = other DNA; note = primer
gtgctggccttggtgagg

SEQ ID NO: 21 - DNA, 20 bp, synthetic construct
  source 1..20: mol_type = other DNA; note = primer
gctgggattgacacaaacac

SEQ ID NO: 22 - DNA, 20 bp, synthetic construct
  source 1..20: mol_type = other DNA; note = primer
aggcaccattgaaagtgtcc

SEQ ID NO: 23 - DNA, 20 bp, synthetic construct
  source 1..20: mol_type = other DNA; note = primer
ttacttacaccccgccagtc

SEQ ID NO: 24 - DNA, 20 bp, synthetic construct
  source 1..20: mol_type = other DNA; note = primer
tatggagtgctgctggtctg

SEQ ID NO: 25 - DNA, 22 bp, synthetic construct
  source 1..22: mol_type = other DNA; note = primer
gttgatatggttcctggcaagc

SEQ ID NO: 26 - DNA, 19 bp, synthetic construct
  source 1..19: mol_type = other DNA; note = primer
ttgccagctccagcagcct

SEQ ID NO: 27 - DNA, 22 bp, synthetic construct
  source 1..22: mol_type = other DNA; note = primer
gatacccctttgacggtaagga

SEQ ID NO: 28 - DNA, 21 bp, synthetic construct
  source 1..21: mol_type = other DNA; note = primer
ccttctcccaaggtccatagc

SEQ ID NO: 29 - DNA, 19 bp, synthetic construct
  source 1..19: mol_type = other DNA; note = primer
ggaccccaaggaaaactgg

SEQ ID NO: 30 - DNA, 22 bp, synthetic construct
  source 1..22: mol_type = other DNA; note = primer
caaccctacaacagacccacac

SEQ ID NO: 31 - DNA, 20 bp, synthetic construct
  source 1..20: mol_type = other DNA; note = primer
tacccccaggagaagattcc

SEQ ID NO: 32 - DNA, 20 bp, synthetic construct
  source 1..20: mol_type = other DNA; note = primer
ttttctgccagtgcctcttt

SEQ ID NO: 33 - DNA, 23 bp, synthetic construct
  source 1..23: mol_type = other DNA; note = primer
ctcagccttttgctcatctcact

SEQ ID NO: 34 - DNA, 25 bp, synthetic construct
  source 1..25: mol_type = other DNA; note = primer
ccaagaggacagactcactttatgg

SEQ ID NO: 35 - DNA, 19 bp, synthetic construct
  source 1..19: mol_type = other DNA; note = primer
cgccttgaagatggcgttg

SEQ ID NO: 36 - DNA, 21 bp, synthetic construct
  source 1..21: mol_type = other DNA; note = primer
gctctggagacttctgaacga

SEQ ID NO: 37 - DNA, 20 bp, synthetic construct
  source 1..20: mol_type = other DNA; note = primer
atggatgaggtggtgaaagc

SEQ ID NO: 38 - DNA, 20 bp, synthetic construct
  source 1..20: mol_type = other DNA; note = primer
cagtgctcacatggctgact

SEQ ID NO: 39 - DNA, 20 bp, synthetic construct
  source 1..20: mol_type = other DNA; note = primer
acccagtttccaccatgatt

SEQ ID NO: 40 - DNA, 20 bp, synthetic construct
  source 1..20: mol_type = other DNA; note = primer
cccaaaatgcaaggaacact

SEQ ID NO: 41 - DNA, 20 bp, synthetic construct
  source 1..20: mol_type = other DNA; note = primer
ccattagaaagcagttccgc

SEQ ID NO: 42 - DNA, 20 bp, synthetic construct
  source 1..20: mol_type = other DNA; note = primer
tgggtaggagatggagatgc

SEQ ID NO: 43 - DNA, 20 bp, synthetic construct
  source 1..20: mol_type = other DNA; note = primer
tcggctttttgccatctgtg

SEQ ID NO: 44 - DNA, 20 bp, synthetic construct
  source 1..20: mol_type = other DNA; note = primer
tgtccaaatgtgccgtgtga